European Patent Application EP 4 616 911 A2, published September 17, 2025. Title: ARGINASE ALBUMIN BINDING DOMAIN FUSION PROTEINS AND METHODS OF USE THEREOF. Applicant: The Hong Kong Polytechnic University. Application EP. The sequence listing filed with the application follows.

SEQUENCE LISTING (113 sequences)

SEQ ID NO: 1 - DNA, 50 bp, synthetic construct
  misc_feature 1..50: note = ABD Primer 1, Synthesized in the Lab
  source 1..50: mol_type = other DNA
ggagatggacatatgcatcatcaccatcaccatgatgaagccgtggatgc

SEQ ID NO: 2 - DNA, 50 bp, synthetic construct
  misc_feature 1..50: note = ABD Primer 2, Synthesized in the Lab
  source 1..50: mol_type = other DNA
gctaagactttagcttcagctaaggaattcgcatccacggcttcatcatg

SEQ ID NO: 3 - DNA, 50 bp, synthetic construct
  misc_feature 1..50: note = ABD Primer 3, Synthesized in the Lab
  source 1..50: mol_type = other DNA
ccttagctgaagctaaagtcttagctaacagagaacttgacaaatatgga

SEQ ID NO: 4 - DNA, 50 bp, synthetic construct
  misc_feature 1..50: note = ABD Primer 4, Synthesized in the Lab
  source 1..50: mol_type = other DNA
taggttcttgtaatagtcacttactccatatttgtcaagttctctgttag

SEQ ID NO: 5 - DNA, 50 bp, synthetic construct
  misc_feature 1..50: note = ABD Primer 5, Synthesized in the Lab
  source 1..50: mol_type = other DNA
ggagtaagtgactattacaagaacctaatcaacaatgccaaaactgttga

SEQ ID NO: 6 - DNA, 50 bp, synthetic construct
  misc_feature 1..50: note = ABD Primer 6, Synthesized in the Lab
  source 1..50: mol_type = other DNA
aaatttcatctatcagtgcttttacaccttcaacagttttggcattgttg

SEQ ID NO: 7 - DNA, 50 bp, synthetic construct
  misc_feature 1..50: note = ABD Primer 7, Synthesized in the Lab
  source 1..50: mol_type = other DNA
gtaaaagcactgatagatgaaattttagctgcattaccttcgggtagtaa

SEQ ID NO: 8 - DNA, 50 bp, synthetic construct
  misc_feature 1..50: note = ABD Primer 8, Synthesized in the Lab
  source 1..50: mol_type = other DNA
tccgccgctaccattgttattattgttgttactacccgaaggtaatgcag

SEQ ID NO: 9 - DNA, 47 bp, synthetic construct
  misc_feature 1..47: note = ABD Primer 9, Synthesized in the Lab
  source 1..47: mol_type = other DNA
gatcttaagcatatgcatcatcaccatcaccatgatgaagcggtgga

SEQ ID NO: 10 - DNA, 47 bp, synthetic construct
  misc_feature 1..47: note = ABD Primer 10, Synthesized in the Lab
  source 1..47: mol_type = other DNA
gcttctttcgcttccgccaggctgttcgcatccaccgcttcatcatg

SEQ ID NO: 11 - DNA, 50 bp, synthetic construct
  misc_feature 1..50: note = ABD Primer 11, Synthesized in the Lab
  source 1..50: mol_type = other DNA
gcggaagcgaaagaagcggcgaacgcggaactggatagctatggcgtgag

SEQ ID NO: 12 - DNA, 50 bp, synthetic construct
  misc_feature 1..50: note = ABD Primer 12, Synthesized in the Lab
  source 1..50: mol_type = other DNA
ttatcaatcaggcgtttataaaaatcgctcacgccatagctatccagttc

SEQ ID NO: 13 - DNA, 50 bp, synthetic construct
  misc_feature 1..50: note = ABD Primer 13, Synthesized in the Lab
  source 1..50: mol_type = other DNA
gatttttataaacgcctgattgataaagcgaaaaccgtggaaggcgtgga

SEQ ID NO: 14 - DNA, 51 bp, synthetic construct
  misc_feature 1..51: note = ABD Primer 14, Synthesized in the Lab
  source 1..51: mol_type = other DNA
cggcagcgccgccagaatcgcatctttcagcgcttccacgccttccacggt

SEQ ID NO: 15 - DNA, 50 bp, synthetic construct
  misc_feature 1..50: note = ABD Primer 15, Synthesized in the Lab
  source 1..50: mol_type = other DNA
ttctggcggcgctgccgtcgggtagtaacaacaataataacaatggtagc

SEQ ID NO: 16 - DNA, 39 bp, synthetic construct
  misc_feature 1..39: note = ABD Primer 16, Synthesized in the Lab
  source 1..39: mol_type = other DNA
ggatccgccgctaccattgttattattgttgttactacc

SEQ ID NO: 17 - DNA, 50 bp, synthetic construct
  misc_feature 1..50: note = ABD Primer 17, Synthesized in the Lab
  source 1..50: mol_type = other DNA
catatgttagctgatggatccagtaacaacaataataacaatggtagcgg

SEQ ID NO: 18 - DNA, 50 bp, synthetic construct
  misc_feature 1..50: note = ABD Primer 18, Synthesized in the Lab
  source 1..50: mol_type = other DNA
aattcgcatccacggcttcatcaccgccgctaccattgttattattgttg

SEQ ID NO: 19 - DNA, 50 bp, synthetic construct
  misc_feature 1..50: note = ABD Primer 19, Synthesized in the Lab
  source 1..50: mol_type = other DNA
gaagccgtggatgcgaattccttagctgaagctaaagtcttagctaacag

SEQ ID NO: 20 - DNA, 50 bp, synthetic construct
  misc_feature 1..50: note = ABD Primer 20, Synthesized in the Lab
  source 1..50: mol_type = other DNA
cttactccatatttgtcaagttctctgttagctaagactttagcttcagc

SEQ ID NO: 21 - DNA, 50 bp, synthetic construct
  misc_feature 1..50: note = ABD Primer 21, Synthesized in the Lab
  source 1..50: mol_type = other DNA
gagaacttgacaaatatggagtaagtgactattacaagaacctaatcaac

SEQ ID NO: 22 - DNA, 50 bp, synthetic construct
  misc_feature 1..50: note = ABD Primer 22, Synthesized in the Lab
  source 1..50: mol_type = other DNA
tacaccttcaacagttttggcattgttgattaggttcttgtaatagtcac

SEQ ID NO: 23 - DNA, 50 bp, synthetic construct
  misc_feature 1..50: note = ABD Primer 23, Synthesized in the Lab
  source 1..50: mol_type = other DNA
gccaaaactgttgaaggtgtaaaagcactgatagatgaaattttagctgc

SEQ ID NO: 24 - DNA, 50 bp, synthetic construct
  misc_feature 1..50: note = ABD Primer 24, Synthesized in the Lab
  source 1..50: mol_type = other DNA
atggtgatggtgatgatgaggtaatgcagctaaaatttcatctatcagtg

SEQ ID NO: 25 - DNA, 50 bp, synthetic construct
  misc_feature 1..50: note = ABD Primer 25, Synthesized in the Lab
  source 1..50: mol_type = other DNA
catatgttatgcgatggatccagtaacaacaataataacaatggtagcgg

SEQ ID NO: 26 - DNA, 50 bp, synthetic construct
  misc_feature 1..50: note = ABD Primer 26, Synthesized in the Lab
  source 1..50: mol_type = other DNA
tgttcgcatccaccgcttcatcaccgccgctaccattgttattattgttg

SEQ ID NO: 27 - DNA, 50 bp, synthetic construct
  misc_feature 1..50: note = ABD Primer 27, Synthesized in the Lab
  source 1..50: mol_type = other DNA
gaagcggtggatgcgaacagcctggcggaagcgaaagaagcggcgaacgc

SEQ ID NO: 28 - DNA, 50 bp, synthetic construct
  misc_feature 1..50: note = ABD Primer 28, Synthesized in the Lab
  source 1..50: mol_type = other DNA
aaaatcgctcacgccatagctatccagttccgcgttcgccgcttctttcg

SEQ ID NO: 29 - DNA, 50 bp, synthetic construct
  misc_feature 1..50: note = ABD Primer 29, Synthesized in the Lab
  source 1..50: mol_type = other DNA
ctatggcgtgagcgatttttataaacgcctgattgataaagcgaaaaccg

SEQ ID NO: 30 - DNA, 50 bp, synthetic construct
  misc_feature 1..50: note = ABD Primer 30, Synthesized in the Lab
  source 1..50: mol_type = other DNA
tcgcatctttcagcgcttccacgccttccacggttttcgctttatcaatc

SEQ ID NO: 31 - DNA, 50 bp, synthetic construct
  misc_feature 1..50: note = ABD Primer 31, Synthesized in the Lab
  source 1..50: mol_type = other DNA
gaagcgctgaaagatgcgattctggcggcgctgccgcatcatcaccatca

SEQ ID NO: 32 - DNA, 35 bp, synthetic construct
  misc_feature 1..35: note = ABD Primer 32, Synthesized in the Lab
  source 1..35: mol_type = other DNA
ctaaaagcttaatggtgatggtgatgatgcggcag

SEQ ID NO: 33 - DNA, 222 bp, synthetic construct
  misc_feature 1..222: note = His-ABD-Linker, Synthesized in the Lab
  source 1..222: mol_type = other DNA
atgcatcatcaccatcaccatgatgaagccgtggatgcgaattccttagctgaagctaaagtcttagctaacagagaacttgacaaatatggagtaagtgactattacaagaacctaatcaacaatgccaaaactgttgaaggtgtaaaagcactgatagatgaaattttagctgcattaccttcgggtagtaacaacaataataacaatggtagcggcgga

SEQ ID NO: 34 - DNA, 222 bp, synthetic construct
  misc_feature 1..222: note = His-ABD094-Linker, Synthesized in the Lab
  source 1..222: mol_type = other DNA
atgcatcatcaccatcaccatgatgaagcggtggatgcgaacagcctggcggaagcgaaagaagcggcgaacgcggaactggatagctatggcgtgagcgatttttataaacgcctgattgataaagcgaaaaccgtggaaggcgtggaagcgctgaaagatgcgattctggcggcgctgccgtcgggtagtaacaacaataataacaatggtagcggcgga

SEQ ID NO: 35 - DNA, 222 bp, synthetic construct
  misc_feature 1..222: note = Linker-ABD-His, Synthesized in the Lab
  source 1..222: mol_type = other DNA
ggatccagtaacaacaataataacaatggtagcggcggtgatgaagccgtggatgcgaattccttagctgaagctaaagtcttagctaacagagaacttgacaaatatggagtaagtgactattacaagaacctaatcaacaatgccaaaactgttgaaggtgtaaaagcactgatagatgaaattttagctgcattacctcatcatcaccatcaccattaa

SEQ ID NO: 36 - DNA, 222 bp, synthetic construct
  misc_feature 1..222: note = Linker-ABD094-His, Synthesized in the Lab
  source 1..222: mol_type = other DNA
ggatccagtaacaacaataataacaatggtagcggcggtgatgaagcggtggatgcgaacagcctggcggaagcgaaagaagcggcgaacgcggaactggatagctatggcgtgagcgatttttataaacgcctgattgataaagcgaaaaccgtggaaggcgtggaagcgctgaaagatgcgattctggcggcgctgccgcatcatcaccatcaccattaa

SEQ ID NO: 37 - DNA, 1191 bp, synthetic construct
  misc_feature 1..1191: note = N-ABD-rhArg gene, Synthesized in the Lab
  source 1..1191: mol_type = other DNA
atgcatcatcaccatcaccatgatgaagccgtggatgcgaattccttagctgaagctaaagtcttagctaacagagaacttgacaaatatggagtaagtgactattacaagaacctaatcaacaatgccaaaactgttgaaggtgtaaaagcactgatagatgaaattttagctgcattaccttcgggtagtaacaacaataataacaatggtagcggcggaatgtccgccaagtccagaaccatagggattattggagctcctttctcaaagggacagccacgaggaggggtggaagaaggccctacagtattgagaaaggctggtctgcttgagaaacttaaagaacaagagtgtgatgtgaaggattatggggacctgccctttgctgacatccctaatgacagtccctttcaaattgtgaagaatccaaggtctgtgggaaaagcaagcgagcagctggctggcaaggtggcagaagtcaagaagaacggaagaatcagcctggtgctgggcggagaccacagtttggcaattggaagcatctctggccatgccagggtccaccctgatcttggagtcatctgggtggatgctcacactgatatcaacactccactgacaaccacaagtggaaacttgcatggacaacctgtatctttcctcctgaaggaactaaaaggaaagattcccgatgtgccaggattctcctgggtgactccctgtatatctgccaaggatattgtgtatattggcttgagagacgtggaccctggggaacactacattttgaaaactctaggcattaaatacttttcaatgactgaagtggacagactaggaattggcaaggtgatggaagaaacactcagctatctactaggaagaaagaaaaggccaattcatctaagttttgatgttgacggactggacccatctttcacaccagctactggcacaccagtcgtgggaggtctgacatacagagaaggtctctacatcacagaagaaatctacaaaacagggctactctcaggattagatataatggaagtgaacccatccctggggaagacaccagaagaagtaactcgaacagtgaacacagcagttgcaataaccttggcttgtttcggacttgctcgggagggtaatcacaagcctattgactaccttaacccacctaagtaa

SEQ ID NO: 38 - DNA, 1191 bp, synthetic construct
  misc_feature 1..1191: note = N-ABD094-rhArg gene, Synthesized in the Lab
  source 1..1191: mol_type = other DNA
atgcatcatcaccatcaccatgatgaagcggtggatgcgaacagcctggcggaagcgaaagaagcggcgaacgcggaactggatagctatggcgtgagcgatttttataaacgcctgattgataaagcgaaaaccgtggaaggcgtggaagcgctgaaagatgcgattctggcggcgctgccgtcgggtagtaacaacaataataacaatggtagcggcggaatgtccgccaagtccagaaccatagggattattggagctcctttctcaaagggacagccacgaggaggggtggaagaaggccctacagtattgagaaaggctggtctgcttgagaaacttaaagaacaagagtgtgatgtgaaggattatggggacctgccctttgctgacatccctaatgacagtccctttcaaattgtgaagaatccaaggtctgtgggaaaagcaagcgagcagctggctggcaaggtggcagaagtcaagaagaacggaagaatcagcctggtgctgggcggagaccacagtttggcaattggaagcatctctggccatgccagggtccaccctgatcttggagtcatctgggtggatgctcacactgatatcaacactccactgacaaccacaagtggaaacttgcatggacaacctgtatctttcctcctgaaggaactaaaaggaaagattcccgatgtgccaggattctcctgggtgactccctgtatatctgccaaggatattgtgtatattggcttgagagacgtggaccctggggaacactacattttgaaaactctaggcattaaatacttttcaatgactgaagtggacagactaggaattggcaaggtgatggaagaaacactcagctatctactaggaagaaagaaaaggccaattcatctaagttttgatgttgacggactggacccatctttcacaccagctactggcacaccagtcgtgggaggtctgacatacagagaaggtctctacatcacagaagaaatctacaaaacagggctactctcaggattagatataatggaagtgaacccatccctggggaagacaccagaagaagtaactcgaacagtgaacacagcagttgcaataaccttggcttgtttcggacttgctcgggagggtaatcacaagcctattgactaccttaacccacctaagtaa

SEQ ID NO: 39 - DNA, 1188 bp, synthetic construct
  misc_feature 1..1188: note = C-ABD-rhArg gene, Synthesized in the Lab
  source 1..1188: mol_type = other DNA
atgagcgccaagtccagaaccatagggattattggagctcctttctcaaagggacagccacgaggaggggtggaagaaggccctacagtattgagaaaggctggtctgcttgagaaacttaaagaacaagagtgtgatgtgaaggattatggggacctgccctttgctgacatccctaatgacagtccctttcaaattgtgaagaatccaaggtctgtgggaaaagcaagcgagcagctggctggcaaggtggcagaagtcaagaagaacggaagaatcagcctggtgctgggcggagaccacagtttggcaattggaagcatctctggccatgccagggtccaccctgatcttggagtcatctgggtggatgctcacactgatatcaacactccactgacaaccacaagtggaaacttgcatggacaacctgtatctttcctcctgaaggaactaaaaggaaagattcccgatgtgccaggattctcctgggtgactccctgtatatctgccaaggatattgtgtatattggcttgagagacgtggaccctggggaacactacattttgaaaactctaggcattaaatacttttcaatgactgaagtggacagactaggaattggcaaggtgatggaagaaacactcagctatctactaggaagaaagaaaaggccaattcatctaagttttgatgttgacggactggacccatctttcacaccagctactggcacaccagtcgtgggaggtctgacatacagagaaggtctctacatcacagaagaaatctacaaaacagggctactctcaggattagatataatggaagtgaacccatccctggggaagacaccagaagaagtaactcgaacagtgaacacagcagttgcaataaccttggcttgtttcggacttgctcgggagggtaatcacaagcctattgactaccttaacccacctaagggatccagtaacaacaataataacaatggtagcggcggtgatgaagccgtggatgcgaattccttagctgaagctaaagtcttagctaacagagaacttgacaaatatggagtaagtgactattacaagaacctaatcaacaatgccaaaactgttgaaggtgtaaaagcactgatagatgaaattttagctgcattacctcatcatcaccatcaccattaa

SEQ ID NO: 40 - DNA, 1188 bp, synthetic construct
  misc_feature 1..1188: note = C-ABD094-rhArg gene, Synthesized in the Lab
  source 1..1188: mol_type = other DNA
atgagcgccaagtccagaaccatagggattattggagctcctttctcaaagggacagccacgaggaggggtggaagaaggccctacagtattgagaaaggctggtctgcttgagaaacttaaagaacaagagtgtgatgtgaaggattatggggacctgccctttgctgacatccctaatgacagtccctttcaaattgtgaagaatccaaggtctgtgggaaaagcaagcgagcagctggctggcaaggtggcagaagtcaagaagaacggaagaatcagcctggtgctgggcggagaccacagtttggcaattggaagcatctctggccatgccagggtccaccctgatcttggagtcatctgggtggatgctcacactgatatcaacactccactgacaaccacaagtggaaacttgcatggacaacctgtatctttcctcctgaaggaactaaaaggaaagattcccgatgtgccaggattctcctgggtgactccctgtatatctgccaaggatattgtgtatattggcttgagagacgtggaccctggggaacactacattttgaaaactctaggcattaaatacttttcaatgactgaagtggacagactaggaattggcaaggtgatggaagaaacactcagctatctactaggaagaaagaaaaggccaattcatctaagttttgatgttgacggactggacccatctttcacaccagctactggcacaccagtcgtgggaggtctgacatacagagaaggtctctacatcacagaagaaatctacaaaacagggctactctcaggattagatataatggaagtgaacccatccctggggaagacaccagaagaagtaactcgaacagtgaacacagcagttgcaataaccttggcttgtttcggacttgctcgggagggtaatcacaagcctattgactaccttaacccacctaagggatccagtaacaacaataataacaatggtagcggcggtgatgaagcggtggatgcgaacagcctggcggaagcgaaagaagcggcgaacgcggaactggatagctatggcgtgagcgatttttataaacgcctgattgataaagcgaaaaccgtggaaggcgtggaagcgctgaaagatgcgattctggcggcgctgccgcatcatcaccatcaccattaa

SEQ ID NO: 41 - DNA, 1125 bp, synthetic construct
  misc_feature 1..1125: note = N-ABD-BCA gene, Synthesized in the Lab
  source 1..1125: mol_type = other DNA
atgcatcatcaccatcaccatgatgaagccgtggatgcgaattccttagctgaagctaaagtcttagctaacagagaacttgacaaatatggagtaagtgactattacaagaacctaatcaacaatgccaaaactgttgaaggtgtaaaagcactgatagatgaaattttagctgcattaccttcgggtagtaacaacaataataacaatggtagcggcggatccatgaagccaatttcaattatcggggttccgatggatttagggcagacacgccgcggcgttgatatggggccgagcgcaatgcgttatgcaggcgtcatcgaacgtctggaacgtcttcattacgatattgaagatttgggagatattccgattggaaaagcagagcggttgcacgagcaaggagattcacggttgcgcaatttgaaagcggttgcggaagcgaacgagaaacttgcggcggcggttgaccaagtcgttcagcgggggcgatttccgcttgtgttgggcggcgaccatagcatcgccattggcacgctcgccggggtggcgaaacattatgagcggcttggagtgatctggtatgacgcgcatggcgacgtcaacaccgcggaaacgtcgccgtctggaaacattcatggcatgccgctggcggcgagcctcgggtttggccatccggcgctgacgcaaatcggcggatacagccccaaaatcaagccggaacatgtcgtgttgatcggcgtccgttcccttgatgaaggggagaagaagtttattcgcgaaaaaggaatcaaaatttacacgatgcatgaggttgatcggctcggaatgacaagggtgatggaagaaacgatcgcctatttaaaagaacgaacggatggcgttcatttgtcgcttgacttggatggccttgacccaagcgacgcaccgggagtcggaacgcctgtcattggaggattgacataccgcgaaagccatttggcgatggagatgctggccgaggcacaaatcatcacttcagcggaatttgtcgaagtgaacccgatcttggatgagcggaacaaaacagcatcagtggctgtagcgctgatggggtcgttgtttggtgaaaaactcatgtaa

SEQ ID NO: 42 - DNA, 1125 bp, synthetic construct
  misc_feature 1..1125: note = N-ABD094-BCA gene, Synthesized in the Lab
  source 1..1125: mol_type = other DNA
atgcatcatcaccatcaccatgatgaagcggtggatgcgaacagcctggcggaagcgaaagaagcggcgaacgcggaactggatagctatggcgtgagcgatttttataaacgcctgattgataaagcgaaaaccgtggaaggcgtggaagcgctgaaagatgcgattctggcggcgctgccgtcgggtagtaacaacaataataacaatggtagcggcggatccatgaagccaatttcaattatcggggttccgatggatttagggcagacacgccgcggcgttgatatggggccgagcgcaatgcgttatgcaggcgtcatcgaacgtctggaacgtcttcattacgatattgaagatttgggagatattccgattggaaaagcagagcggttgcacgagcaaggagattcacggttgcgcaatttgaaagcggttgcggaagcgaacgagaaacttgcggcggcggttgaccaagtcgttcagcgggggcgatttccgcttgtgttgggcggcgaccatagcatcgccattggcacgctcgccggggtggcgaaacattatgagcggcttggagtgatctggtatgacgcgcatggcgacgtcaacaccgcggaaacgtcgccgtctggaaacattcatggcatgccgctggcggcgagcctcgggtttggccatccggcgctgacgcaaatcggcggatacagccccaaaatcaagccggaacatgtcgtgttgatcggcgtccgttcccttgatgaaggggagaagaagtttattcgcgaaaaaggaatcaaaatttacacgatgcatgaggttgatcggctcggaatgacaagggtgatggaagaaacgatcgcctatttaaaagaacgaacggatggcgttcatttgtcgcttgacttggatggccttgacccaagcgacgcaccgggagtcggaacgcctgtcattggaggattgacataccgcgaaagccatttggcgatggagatgctggccgaggcacaaatcatcacttcagcggaatttgtcgaagtgaacccgatcttggatgagcggaacaaaacagcatcagtggctgtagcgctgatggggtcgttgtttggtgaaaaactcatgtaa

SEQ ID NO: 43 - DNA, 1119 bp, synthetic construct
  misc_feature 1..1119: note = C-ABD-BCA gene, Synthesized in the Lab
  source 1..1119: mol_type = other DNA
atgaagccaatttcaattatcggggttccgatggatttagggcagacacgccgcggcgttgatatggggccgagcgcaatgcgttatgcaggcgtcatcgaacgtctggaacgtcttcattacgatattgaagatttgggagatattccgattggaaaagcagagcggttgcacgagcaaggagattcacggttgcgcaatttgaaagcggttgcggaagcgaacgagaaacttgcggcggcggttgaccaagtcgttcagcgggggcgatttccgcttgtgttgggcggcgaccatagcatcgccattggcacgctcgccggggtggcgaaacattatgagcggcttggagtgatctggtatgacgcgcatggcgacgtcaacaccgcggaaacgtcgccgtctggaaacattcatggcatgccgctggcggcgagcctcgggtttggccatccggcgctgacgcaaatcggcggatacagccccaaaatcaagccggaacatgtcgtgttgatcggcgtccgttcccttgatgaaggggagaagaagtttattcgcgaaaaaggaatcaaaatttacacgatgcatgaggttgatcggctcggaatgacaagggtgatggaagaaacgatcgcctatttaaaagaacgaacggatggcgttcatttgtcgcttgacttggatggccttgacccaagcgacgcaccgggagtcggaacgcctgtcattggaggattgacataccgcgaaagccatttggcgatggagatgctggccgaggcacaaatcatcacttcagcggaatttgtcgaagtgaacccgatcttggatgagcggaacaaaacagcatcagtggctgtagcgctgatggggtcgttgtttggtgaaaaactcatgggatccagtaacaacaataataacaatggtagcggcggtgatgaagccgtggatgcgaattccttagctgaagctaaagtcttagctaacagagaacttgacaaatatggagtaagtgactattacaagaacctaatcaacaatgccaaaactgttgaaggtgtaaaagcactgatagatgaaattttagctgcattacctcatcatcaccatcaccattaa

SEQ ID NO: 44 - DNA, 1119 bp, synthetic construct
  misc_feature 1..1119: note = C-ABD094-BCA gene, Synthesized in the Lab
  source 1..1119: mol_type = other DNA
atgaagccaatttcaattatcggggttccgatggatttagggcagacacgccgcggcgttgatatggggccgagcgcaatgcgttatgcaggcgtcatcgaacgtctggaacgtcttcattacgatattgaagatttgggagatattccgattggaaaagcagagcggttgcacgagcaaggagattcacggttgcgcaatttgaaagcggttgcggaagcgaacgagaaacttgcggcggcggttgaccaagtcgttcagcgggggcgatttccgcttgtgttgggcggcgaccatagcatcgccattggcacgctcgccggggtggcgaaacattatgagcggcttggagtgatctggtatgacgcgcatggcgacgtcaacaccgcggaaacgtcgccgtctggaaacattcatggcatgccgctggcggcgagcctcgggtttggccatccggcgctgacgcaaatcggcggatacagccccaaaatcaagccggaacatgtcgtgttgatcggcgtccgttcccttgatgaaggggagaagaagtttattcgcgaaaaaggaatcaaaatttacacgatgcatgaggttgatcggctcggaatgacaagggtgatggaagaaacgatcgcctatttaaaagaacgaacggatggcgttcatttgtcgcttgacttggatggccttgacccaagcgacgcaccgggagtcggaacgcctgtcattggaggattgacataccgcgaaagccatttggcgatggagatgctggccgaggcacaaatcatcacttcagcggaatttgtcgaagtgaacccgatcttggatgagcggaacaaaacagcatcagtggctgtagcgctgatggggtcgttgtttggtgaaaaactcatgggatccagtaacaacaataataacaatggtagcggcggtgatgaagcggtggatgcgaacagcctggcggaagcgaaagaagcggcgaacgcggaactggatagctatggcgtgagcgatttttataaacgcctgattgataaagcgaaaaccgtggaaggcgtggaagcgctgaaagatgcgattctggcggcgctgccgcatcatcaccatcaccattaa

SEQ ID NO: 45 - protein, 74 aa, synthetic construct
  REGION 1..74: note = His-ABD-Linker, Synthesized in the Lab
MHHHHHHDEAVDANSLAEAKVLANRELDKYGVSDYYKNLINNAKTVEGVKALIDEILAALPSGSNNNNNNGSGG

SEQ ID NO: 46 - protein, 74 aa, synthetic construct
  REGION 1..74: note = His-ABD094-Linker, Synthesized in the Lab
MHHHHHHDEAVDANSLAEAKEAANAELDSYGVSDFYKRLIDKAKTVEGVEALKDAILAALPSGSNNNNNNGSGG

SEQ ID NO: 47 - protein, 73 aa, synthetic construct
  REGION 1..73: note = Linker-ABD-His, Synthesized in the Lab
GSSNNNNNNGSGGDEAVDANSLAEAKVLANRELDKYGVSDYYKNLINNAKTVEGVKALIDEILAALPHHHHHH

SEQ ID NO: 48 - protein, 73 aa, synthetic construct
  REGION 1..73: note = Linker-ABD094-His, Synthesized in the Lab
GSSNNNNNNGSGGDEAVDANSLAEAKEAANAELDSYGVSDFYKRLIDKAKTVEGVEALKDAILAALPHHHHHH

SEQ ID NO: 49 - protein, 396 aa, synthetic construct
  REGION 1..396: note = N-ABD-rhArg, Synthesized in the Lab
MHHHHHHDEAVDANSLAEAKVLANRELDKYGVSDYYKNLINNAKTVEGVKALIDEILAALPSGSNNNNNNGSGGMSAKSRTIGIIGAPFSKGQPRGGVEEGPTVLRKAGLLEKLKEQECDVKDYGDLPFADIPNDSPFQIVKNPRSVGKASEQLAGKVAEVKKNGRISLVLGGDHSLAIGSISGHARVHPDLGVIWVDAHTDINTPLTTTSGNLHGQPVSFLLKELKGKIPDVPGFSWVTPCISAKDIVYIGLRDVDPGEHYILKTLGIKYFSMTEVDRLGIGKVMEETLSYLLGRKKRPIHLSFDVDGLDPSFTPATGTPVVGGLTYREGLYITEEIYKTGLLSGLDIMEVNPSLGKTPEEVTRTVNTAVAITLACFGLAREGNHKPIDYLNPPK

SEQ ID NO: 50 - protein, 396 aa, synthetic construct
  REGION 1..396: note = N-ABD094-rhArg, Synthesized in the Lab
MHHHHHHDEAVDANSLAEAKEAANAELDSYGVSDFYKRLIDKAKTVEGVEALKDAILAALPSGSNNNNNNGSGGMSAKSRTIGIIGAPFSKGQPRGGVEEGPTVLRKAGLLEKLKEQECDVKDYGDLPFADIPNDSPFQIVKNPRSVGKASEQLAGKVAEVKKNGRISLVLGGDHSLAIGSISGHARVHPDLGVIWVDAHTDINTPLTTTSGNLHGQPVSFLLKELKGKIPDVPGFSWVTPCISAKDIVYIGLRDVDPGEHYILKTLGIKYFSMTEVDRLGIGKVMEETLSYLLGRKKRPIHLSFDVDGLDPSFTPATGTPVVGGLTYREGLYITEEIYKTGLLSGLDIMEVNPSLGKTPEEVTRTVNTAVAITLACFGLAREGNHKPIDYLNPPK

SEQ ID NO: 51 - protein, 395 aa, synthetic construct
  REGION 1..395: note = C-ABD-rhArg, Synthesized in the Lab
MSAKSRTIGIIGAPFSKGQPRGGVEEGPTVLRKAGLLEKLKEQECDVKDYGDLPFADIPNDSPFQIVKNPRSVGKASEQLAGKVAEVKKNGRISLVLGGDHSLAIGSISGHARVHPDLGVIWVDAHTDINTPLTTTSGNLHGQPVSFLLKELKGKIPDVPGFSWVTPCISAKDIVYIGLRDVDPGEHYILKTLGIKYFSMTEVDRLGIGKVMEETLSYLLGRKKRPIHLSFDVDGLDPSFTPATGTPVVGGLTYREGLYITEEIYKTGLLSGLDIMEVNPSLGKTPEEVTRTVNTAVAITLACFGLAREGNHKPIDYLNPPKGSSNNNNNNGSGGDEAVDANSLAEAKVLANRELDKYGVSDYYKNLINNAKTVEGVKALIDEILAALPHHHHHH

SEQ ID NO: 52 - protein, 395 aa, synthetic construct
  REGION 1..395: note = C-ABD094-rhArg, Synthesized in the Lab
MSAKSRTIGIIGAPFSKGQPRGGVEEGPTVLRKAGLLEKLKEQECDVKDYGDLPFADIPNDSPFQIVKNPRSVGKASEQLAGKVAEVKKNGRISLVLGGDHSLAIGSISGHARVHPDLGVIWVDAHTDINTPLTTTSGNLHGQPVSFLLKELKGKIPDVPGFSWVTPCISAKDIVYIGLRDVDPGEHYILKTLGIKYFSMTEVDRLGIGKVMEETLSYLLGRKKRPIHLSFDVDGLDPSFTPATGTPVVGGLTYREGLYITEEIYKTGLLSGLDIMEVNPSLGKTPEEVTRTVNTAVAITLACFGLAREGNHKPIDYLNPPKGSSNNNNNNGSGGDEAVDANSLAEAKEAANAELDSYGVSDFYKRLIDKAKTVEGVEALKDAILAALPHHHHHH

SEQ ID NO: 53 - protein, 374 aa, synthetic construct
  REGION 1..374: note = N-ABD-BCA, Synthesized in the Lab
MHHHHHHDEAVDANSLAEAKVLANRELDKYGVSDYYKNLINNAKTVEGVKALIDEILAALPSGSNNNNNNGSGGSMKPISIIGVPMDLGQTRRGVDMGPSAMRYAGVIERLERLHYDIEDLGDIPIGKAERLHEQGDSRLRNLKAVAEANEKLAAAVDQVVQRGRFPLVLGGDHSIAIGTLAGVAKHYERLGVIWYDAHGDVNTAETSPSGNIHGMPLAASLGFGHPALTQIGGYSPKIKPEHVVLIGVRSLDEGEKKFIREKGIKIYTMHEVDRLGMTRVMEETIAYLKERTDGVHLSLDLDGLDPSDAPGVGTPVIGGLTYRESHLAMEMLAEAQIITSAEFVEVNPILDERNKTASVAVALMGSLFGEKLM

SEQ ID NO: 54 - protein, 374 aa, synthetic construct
  REGION 1..374: note = N-ABD094-BCA, Synthesized in the Lab
MHHHHHHDEAVDANSLAEAKEAANAELDSYGVSDFYKRLIDKAKTVEGVEALKDAILAALPSGSNNNNNNGSGGSMKPISIIGVPMDLGQTRRGVDMGPSAMRYAGVIERLERLHYDIEDLGDIPIGKAERLHEQGDSRLRNLKAVAEANEKLAAAVDQVVQRGRFPLVLGGDHSIAIGTLAGVAKHYERLGVIWYDAHGDVNTAETSPSGNIHGMPLAASLGFGHPALTQIGGYSPKIKPEHVVLIGVRSLDEGEKKFIREKGIKIYTMHEVDRLGMTRVMEETIAYLKERTDGVHLSLDLDGLDPSDAPGVGTPVIGGLTYRESHLAMEMLAEAQIITSAEFVEVNPILDERNKTASVAVALMGSLFGEKLM

SEQ ID NO: 55 - protein, 372 aa, synthetic construct
  REGION 1..372: note = C-ABD-BCA, Synthesized in the Lab
MKPISIIGVPMDLGQTRRGVDMGPSAMRYAGVIERLERLHYDIEDLGDIPIGKAERLHEQGDSRLRNLKAVAEANEKLAAAVDQVVQRGRFPLVLGGDHSIAIGTLAGVAKHYERLGVIWYDAHGDVNTAETSPSGNIHGMPLAASLGFGHPALTQIGGYSPKIKPEHVVLIGVRSLDEGEKKFIREKGIKIYTMHEVDRLGMTRVMEETIAYLKERTDGVHLSLDLDGLDPSDAPGVGTPVIGGLTYRESHLAMEMLAEAQIITSAEFVEVNPILDERNKTASVAVALMGSLFGEKLMGSSNNNNNNGSGGDEAVDANSLAEAKVLANRELDKYGVSDYYKNLINNAKTVEGVKALIDEILAALPHHHHHH

SEQ ID NO: 56 - protein, 372 aa, synthetic construct
  REGION 1..372: note = C-ABD094-BCA, Synthesized in the Lab
MKPISIIGVPMDLGQTRRGVDMGPSAMRYAGVIERLERLHYDIEDLGDIPIGKAERLHEQGDSRLRNLKAVAEANEKLAAAVDQVVQRGRFPLVLGGDHSIAIGTLAGVAKHYERLGVIWYDAHGDVNTAETSPSGNIHGMPLAASLGFGHPALTQIGGYSPKIKPEHVVLIGVRSLDEGEKKFIREKGIKIYTMHEVDRLGMTRVMEETIAYLKERTDGVHLSLDLDGLDPSDAPGVGTPVIGGLTYRESHLAMEMLAEAQIITSAEFVEVNPILDERNKTASVAVALMGSLFGEKLMGSSNNNNNNGSGGDEAVDANSLAEAKEAANAELDSYGVSDFYKRLIDKAKTVEGVEALKDAILAALPHHHHHH

SEQ ID NO: 57 - DNA, 50 bp, synthetic construct
  misc_feature 1..50: note = ABD094-0F Primer, Synthesized in the Lab
  source 1..50: mol_type = other DNA
attctggcagcgctgccgtcgggtagtaacaacaataataacaatggtag

SEQ ID NO: 58 - DNA, 50 bp, synthetic construct
  misc_feature 1..50: note = ABD094-1F Primer, Synthesized in the Lab
  source 1..50: mol_type = other DNA
aaccgtggaaggtgtggaagcgctgaaagatgcgattctggcagcgctgc

SEQ ID NO: 59 - DNA, 50 bp, synthetic construct
  misc_feature 1..50: note = ABD094-2F Primer, Synthesized in the Lab
  source 1..50: mol_type = other DNA
gatttttataaacgtctgattgataaagcgaaaaccgtggaaggtgtgga

SEQ ID NO: 60 - DNA, 50 bp, synthetic construct
  misc_feature 1..50: note = ABD094-3F Primer, Synthesized in the Lab
  source 1..50: mol_type = other DNA
ctggatagctatggcgtgagcgatttttataaacgtctgattgataaagc

SEQ ID NO: 61 - DNA, 50 bp, synthetic construct
  misc_feature 1..50: note = ABD094-4F Primer, Synthesized in the Lab
  source 1..50: mol_type = other DNA
gcggaagcgaaagaagcagcaaacgcggaactggatagctatggcgtgag

SEQ ID NO: 62 - DNA, 50 bp, synthetic construct
  misc_feature 1..50: note = ABD094-5F Primer, Synthesized in the Lab
  source 1..50: mol_type = other DNA
accatgatgaagccgtggatgcgaattccctggcggaagcgaaagaagca

SEQ ID NO: 63 - DNA, 46 bp, synthetic construct
  misc_feature 1..46: note = abdNde-F Primer, Synthesized in the Lab
  source 1..46: mol_type = other DNA
ggagatatacatatgcatcatcaccatcaccatgatgaagccgtgg

SEQ ID NO: 64 - DNA, 42 bp, synthetic construct
  misc_feature 1..42: note = HuArgHinBam-R Primer, Synthesized in the Lab
  source 1..42: mol_type = other DNA
tgactaccttaacccacctaagtaagcttggatcctgtaacg

SEQ ID NO: 65 - DNA, 1220 bp, synthetic construct
  misc_feature 1..1220: note = N-ABD094-rhArg gene, Synthesized in the Lab
  source 1..1220: mol_type = other DNA
ggagatatacatatgcatcatcaccatcaccatgatgaagccgtggatgcgaattccctggcggaagcgaaagaagcagcaaacgcggaactggatagctatggcgtgagcgatttttataaacgtctgattgataaagcgaaaaccgtggaaggtgtggaagcgctgaaagatgcgattctggcagcgctgccgtcgggtagtaacaacaataataacaatggtagcggcggtatgagcgccaagtccagaaccatagggattattggagctcctttctcaaagggacagccacgaggaggggtggaagaaggccctacagtattgagaaaggctggtctgcttgagaaacttaaagaacaagagtgtgatgtgaaggattatggggacctgccctttgctgacatccctaatgacagtccctttcaaattgtgaagaatccaaggtctgtgggaaaagcaagcgagcagctggctggcaaggtggcagaagtcaagaagaacggaagaatcagcctggtgctgggcggagaccacagtttggcaattggaagcatctctggccatgccagggtccaccctgatcttggagtcatctgggtggatgctcacactgatatcaacactccactgacaaccacaagtggaaacttgcatggacaacctgtatctttcctcctgaaggaactaaaaggaaagattcccgatgtgccaggattctcctgggtgactccctgtatatctgccaaggatattgtgtatattggcttgagagacgtggaccctggggaacactacattttgaaaactctaggcattaaatacttttcaatgactgaagtggacagactaggaattggcaaggtgatggaagaaacactcagctatctactaggaagaaagaaaaggccaattcatctaagttttgatgttgacggactggacccatctttcacaccagctactggcacaccagtcgtgggaggtctgacatacagagaaggtctctacatcacagaagaaatctacaaaacagggctactctcaggattagatataatggaagtgaacccatccctggggaagacaccagaagaagtaactcgaacagtgaacacagcagttgcaataaccttggcttgtttcggacttgctcgggagggtaatcacaagcctattgactaccttaacccacctaagtaagcttggatcctgtaacg

SEQ ID NO: 66 - protein, 54 aa, synthetic construct
  REGION 1..54: note = ABD based on Streptococcus sp. G148, Synthesized in the Lab
DEAVDANSLAEAKVLANRELDKYGVSDYYKNLINNAKTVEGVKALIDEILAALP

SEQ ID NO: 67 - protein, 57 aa, synthetic construct
  REGION 1..57: note = ABD based on Streptococcus sp. G148, Synthesized in the Lab
AQHDEAVDANSLAEAKVLANRELDKYGVSDYYKNLINNAKTVEGVKALIDEILAALP

SEQ ID NO: 68 - protein, 46 aa, synthetic construct
  REGION 1..46: note = ABD094 Without Linker, Synthesized in Lab
LAEAKEAANAELDSYGVSDFYKRLIDKAKTVEGVEALKDAILAALP

SEQ ID NO: 69 - protein, 324 aa, Homo sapiens
  SITE 1: note = Xaa - Xaa at position one is either methionine or not present.
XAASAKSRTIGIIGAPFSKGQPRGGVEEGPTVLRKAGLLEKLKEQECDVKDYGDLPFADIPNDSPFQIVKNPRSVGKASEQLAGKVAEVKKNGRISLVLGGDHSLAIGSISGHARVHPDLGVIWVDAHTDINTPLTTTSGNLHGQPVSFLLKELKGKIPDVPGFSWVTPCISAKDIVYIGLRDVDPGEHYILKTLGIKYFSMTEVDRLGIGKVMEETLSYLLGRKKRPIHLSFDVDGLDPSFTPATGTPVVGGLTYREGLYITEEIYKTGLLSGLDIMEVNPSLGKTPEEVTRTVNTAVAITLACFGLAREGNHKPIDYLNPPK

SEQ ID NO: 70 - protein, 299 aa, Bacillus caldovelox
MKPISIIGVPMDLGQTRRGVDMGPSAMRYAGVIERLERLHYDIEDLGDIPIGKAERLHEQGDSRLRNLKAVAEANEKLAAAVDQVVQRGRFPLVLGGDHSIAIGTLAGVAKHYERLGVIWYDAHGDVNTAETSPSGNIHGMPLAASLGFGHPALTQIGGYSPKIKPEHVVLIGVRSLDEGEKKFIREKGIKIYTMHEVDRLGMTRVMEETIAYLKERTDGVHLSLDLDGLDPSDAPGVGTPVIGGLTYRESHLAMEMLAEAQIITSAEFVEVNPILDERNKTASVAVALMGSLFGEKLM

SEQ ID NO: 71 - protein, 299 aa, synthetic construct
  REGION 1..299: note = BCA (S161C) Arginase, Synthesized in the Lab
MKPISIIGVPMDLGQTRRGVDMGPSAMRYAGVIERLERLHYDIEDLGDIPIGKAERLHEQGDSRLRNLKAVAEANEKLAAAVDQVVQRGRFPLVLGGDHSIAIGTLAGVAKHYERLGVIWYDAHGDVNTAETSPSGNIHGMPLAASLGFGHPALTQIGGYCPKIKPEHVVLIGVRSLDEGEKKFIREKGIKIYTMHEVDRLGMTRVMEETIAYLKERTDGVHLSLDLDGLDPSDAPGVGTPVIGGLTYRESHLAMEMLAEAQIITSAEFVEVNPILDERNKTASVAVALMGSLFGEKLM

SEQ ID NO: 72 - protein, 299 aa, synthetic construct
  REGION 1..299: note = BCA (V20P, S161C) Arginase, Synthesized in the Lab
MKPISIIGVPMDLGQTRRGPDMGPSAMRYAGVIERLERLHYDIEDLGDIPIGKAERLHEQGDSRLRNLKAVAEANEKLAAAVDQVVQRGRFPLVLGGDHSIAIGTLAGVAKHYERLGVIWYDAHGDVNTAETSPSGNIHGMPLAASLGFGHPALTQIGGYCPKIKPEHVVLIGVRSLDEGEKKFIREKGIKIYTMHEVDRLGMTRVMEETIAYLKERTDGVHLSLDLDGLDPSDAPGVGTPVIGGLTYRESHLAMEMLAEAQIITSAEFVEVNPILDERNKTASVAVALMGSLFGEKLM

SEQ ID NO: 73 - protein, 12 aa, synthetic construct
  REGION 1..12: note = Linker Sequence 1, Synthesized in the Lab
GSNNNNNNGSGG

SEQ ID NO: 74 - protein, 13 aa, synthetic construct
  REGION 1..13: note = Linker Sequence 2, Synthesized in the Lab
SGSNNNNNNGSGG

SEQ ID NO: 75 - protein, 362 aa, synthetic construct
  REGION 1..362: note = BHA Fusion Protein, Synthesized in the Lab
MKPISIIGVPMDLGQTRRGPDMGPSAMRYAGVIERLERLHYDIEDLGDIPIGKAERLHEQGDSRLRNLKAVAEANEKLAAAVDQVVQRGRFPLVLGGDHSIAIGTLAGVAKHYERLGVIWYDAHGDVNTAETSPSGNIHGMPLAASLGFGHPALTQIGGYCPKIKPEHVVLIGVRSLDEGEKKFIREKGIKIYTMHEVDRLGMTRVMEETIAYLKERTDGVHLSLDLDGLDPSDAPGVGTPVIGGLTYRESHLAMEMLAEAQIITSAEFVEVNPILDERNKTASVAVALMGSLFGEKLMHHHHHHAQHDEAVDANSLAEAKVLANRELDKYGVSDYYKNLINNAKTVEGVKALIDEILAALP

SEQ ID NO: 76 - protein, 362 aa, synthetic construct
  REGION 1..362: note = BAH Fusion Protein, Synthesized in the Lab
MKPISIIGVPMDLGQTRRGPDMGPSAMRYAGVIERLERLHYDIEDLGDIPIGKAERLHEQGDSRLRNLKAVAEANEKLAAAVDQVVQRGRFPLVLGGDHSIAIGTLAGVAKHYERLGVIWYDAHGDVNTAETSPSGNIHGMPLAASLGFGHPALTQIGGYCPKIKPEHVVLIGVRSLDEGEKKFIREKGIKIYTMHEVDRLGMTRVMEETIAYLKERTDGVHLSLDLDGLDPSDAPGVGTPVIGGLTYRESHLAMEMLAEAQIITSAEFVEVNPILDERNKTASVAVALMGSLFGEKLMAQHDEAVDANSLAEAKVLANRELDKYGVSDYYKNLINNAKTVEGVKALIDEILAALPHHHHHH

SEQ ID NO: 77 - DNA, 103 bp, synthetic construct
  misc_feature 1..103: note = 5'-Sense-ABD Primer, Synthesized in Lab
  source 1..103: mol_type = other DNA
gcgcagcatgatgaagccgtggatgcgaacagcttagctgaagctaaagtcttagctaacagagaacttgacaaatatggagtaagtgactattacaagaacc

SEQ ID NO: 78 - DNA, 98 bp, synthetic construct
  misc_feature 1..98: note = 5'-Anti-sense-ABD Primer, Synthesized in the Lab
  source 1..98: mol_type = other DNA
ttaaggtaatgcagctaaaatttcatctatcagtgcttttacaccttcaacagttttggcattgttgattaggttcttgtaatagtcacttactccat

SEQ ID NO: 79 - DNA, 35 bp, synthetic construct
  misc_feature 1..35: note = Forward Primer for Cloning ABD, Synthesized in the Lab
  source 1..35: mol_type = other DNA
gcatcaccatcaccatcacgcgcagcatgatgaag

SEQ ID NO: 80 - DNA, 38 bp, synthetic construct
  misc_feature 1..38: note = Reverse Primer for Cloning ABD, Synthesized in the Lab
  source 1..38: mol_type = other DNA
cgggatccttaaggtaatgcagctaaaatttcatctat

SEQ ID NO: 81 - DNA, 33 bp, synthetic construct
  misc_feature 1..33: note = Forward Primer for Cloning BCA, Synthesized in the Lab
  source 1..33: mol_type = other DNA
ggaattcccatatgaagccaatttcaattatcg

SEQ ID NO: 82 - DNA, 20 bp, synthetic construct
  misc_feature 1..20: note = Reverse Primer for Cloning BCA, Synthesized in the Lab
  source 1..20: mol_type = other DNA
gtgatggtgatggtgatgca

SEQ ID NO: 83 - DNA, 33 bp, synthetic construct; identical to SEQ ID NO: 81
  misc_feature 1..33: note = Forward Primer for Cloning BHA, Synthesized in the Lab
  source 1..33: mol_type = other DNA

SEQ ID NO: 84 - DNA, 38 bp, synthetic construct; identical to SEQ ID NO: 80
  misc_feature 1..38: note = Reverse Primer for Cloning BHA, Synthesized in the Lab
  source 1..38: mol_type = other DNA

SEQ ID NO: 85 - DNA, 39 bp, synthetic construct
  misc_feature 1..39: note = Forward Primer for Cloning ABD, Synthesized in the Lab
  source 1..39: mol_type = other DNA
cgttgtttggtgaaaaactcatggcgcagcatgatgaag

SEQ ID NO: 86 - DNA, 56 bp, synthetic construct
  misc_feature 1..56: note = Reverse Primer for Cloning ABD, Synthesized in the Lab
  source 1..56: mol_type = other DNA
cgggatccttagtgatggtgatggtgatgaggtaatgcagctaaaatttcatctat

SEQ ID NO: 87 - DNA, 33 bp, synthetic construct; identical to SEQ ID NO: 81
  misc_feature 1..33: note = Forward Primer for Cloning BAH, Syntesized in the Lab
  source 1..33: mol_type = other DNA

SEQ ID NO: 88 - DNA, 56 bp, synthetic construct; identical to SEQ ID NO: 86
  misc_feature 1..56: note = Reverse Primer for Cloning BAH, Synthesized in the Lab
  source 1..56: mol_type = other DNA

SEQ ID NO: 89 - protein, 305 aa, synthetic construct
  REGION 1..305: note = BCA (S161C) - His, Synthesized in Lab
MKPISIIGVPMDLGQTRRGVDMGPSAMRYAGVIERLERLHYDIEDLGDIPIGKAERLHEQGDSRLRNLKAVAEANEKLAAAVDQVVQRGRFPLVLGGDHSIAIGTLAGVAKHYERLGVIWYDAHGDVNTAETSPSGNIHGMPLAASLGFGHPALTQIGGYCPKIKPEHVVLIGVRSLDEGEKKFIREKGIKIYTMHEVDRLGMTRVMEETIAYLKERTDGVHLSLDLDGLDPSDAPGVGTPVIGGLTYRESHLAMEMLAEAQIITSAEFVEVNPILDERNKTASVAVALMGSLFGEKLMHHHHHH

SEQ ID NO: 90 - DNA, 42 bp, synthetic construct
  misc_feature 1..42: note = N-ABDHind-R Primer, Synthesized in the Lab
  source 1..42: mol_type = other DNA
acagctaaaagcttatcagcctaggatccgccgctaccattg

SEQ ID NO: 91 - DNA, 38 bp, synthetic construct
  misc_feature 1..38: note = C-ABDNde-F Primer, Synthesized in the Lab
  source 1..38: mol_type = other DNA
tagctgatcatatgttatgcgatggatccagtaacaac

SEQ ID NO: 92 - DNA, 33 bp, synthetic construct
  misc_feature 1..33: note = C-ABDHind-R, Synthesized in the Lab
  source 1..33: mol_type = other DNA
gaccctaaaagcttaatggtgatggtgatgatg

SEQ ID NO: 93 - DNA, 34 bp, synthetic construct
  misc_feature 1..34: note = HARGBam-F Primer, Synthesized in the Lab
  source 1..34: mol_type = other DNA
ttagctggggatccgccaagtccagaaccatagg

SEQ ID NO: 94 - DNA, 35 bp, synthetic construct
  misc_feature 1..35: note = HARGHind-R Primer, Synthesized in the Lab
  source 1..35: mol_type = other DNA
gagatcaaagcttacttaggtgggttaaggtagtc

SEQ ID NO: 95 - DNA, 35 bp, synthetic construct
  misc_feature 1..35: note = HARGNde-F, Synthesized in the Lab
  source 1..35: mol_type = other DNA
taggctgcatatgagcgccaagtccagaaccatag

SEQ ID NO: 96 - DNA, 41 bp, synthetic construct
  misc_feature 1..41: note = HARGBam-R Primer, Synthesized in the Lab
  source 1..41: mol_type = other DNA
atcagctaggatcccttaggtgggttaaggtagtcaatagg

SEQ ID NO: 97 - DNA, 36 bp, synthetic construct
  misc_feature 1..36: note = BCABam-F Primer, Synthesized in the Lab
  source 1..36: mol_type = other DNA
atgctagtggatccatgaagccaatttcaattatcg

SEQ ID NO: 98 - DNA, 38 bp, synthetic construct
  misc_feature 1..38: note = BCAHind-R Primer, Synthesized in the Lab
  source 1..38: mol_type = other DNA
tcagcctaaagcttacatgagtttttcaccaaacaacg

SEQ ID NO: 99 - DNA, 35 bp, synthetic construct
  misc_feature 1..35: note = BCANde-F Primer, Synthesized in the Lab
  source 1..35: mol_type = other DNA
atgctagccatatgaagccaatttcaattatcggg

SEQ ID NO: 100 - DNA, 37 bp, synthetic construct
  misc_feature 1..37: note = BCABam-R Primer, Synthesized in the Lab
  source 1..37: mol_type = other DNA
tcagctaaggatcccatgagtttttcaccaaacaacg

SEQ ID NO: 101 - protein, 329 aa, synthetic construct
  REGION 1..329: note = His-rhArg, Synthesized in Lab
MHHHHHHMSAKSRTIGIIGAPFSKGQPRGGVEEGPTVLRKAGLLEKLKEQECDVKDYGDLPFADIPNDSPFQIVKNPRSVGKASEQLAGKVAEVKKNGRISLVLGGDHSLAIGSISGHARVHPDLGVIWVDAHTDINTPLTTTSGNLHGQPVSFLLKELKGKIPDVPGFSWVTPCISAKDIVYIGLRDVDPGEHYILKTLGIKYFSMTEVDRLGIGKVMEETLSYLLGRKKRPIHLSFDVDGLDPSFTPATGTPVVGGLTYREGLYITEEIYKTGLLSGLDIMEVNPSLGKTPEEVTRTVNTAVAITLACFGLAREGNHKPIDYLNPPK

SEQ ID NO: 102 - protein, 329 aa, synthetic construct
  REGION 1..329: note = His-rhArg-mono-Cys, Synthesized in Lab
MHHHHHHMSAKSRTIGIIGAPFSKGQPRGGVEEGPTVLRKAGLLEKLKEQECDVKDYGDLPFADIPNDSPFQIVKNPRSVGKASEQLAGKVAEVKKNGRISLVLGGDHSLAIGSISGHARVHPDLGVIWVDAHTDINTPLTTTSGNLHGQPVSFLLKELKGKIPDVPGFSWVTPSISAKDIVYIGLRDVDPGEHYILKTLGIKYFSMTEVDRLGIGKVMEETLSYLLGRKKRPIHLSFDVDGLDPSFTPATGTPVVGGLTYREGLYITEEIYKTGLLSGLDIMEVNPSLGKTPEEVTRTVNTAVAITLASFGLAREGNHKPIDYLNPPK

SEQ ID NO: 103 - protein, 322 aa, Homo sapiens
MSAKSRTIGIIGAPFSKGQPRGGVEEGPTVLRKAGLLEKLKEQECDVKDYGDLPFADIPNDSPFQIVKNPRSVGKASEQLAGKVAEVKKNGRISLVLGGDHSLAIGSISGHARVHPDLGVIWVDAHTDINTPLTTTSGNLHGQPVSFLLKELKGKIPDVPGFSWVTPCISAKDIVYIGLRDVDPGEHYILKTLGIKYFSMTEVDRLGIGKVMEETLSYLLGRKKRPIHLSFDVDGLDPSFTPATGTPVVGGLTYREGLYITEEIYKTGLLSGLDIMEVNPSLGKTPEEVTRTVNTAVAITLACFGLAREGNHKPIDYLNPPK

SEQ ID NO: 104 - protein, 322 aa, synthetic construct
  REGION 1..322: note = rhArg-mono-Cys, Synthesized in the Lab
MSAKSRTIGIIGAPFSKGQPRGGVEEGPTVLRKAGLLEKLKEQECDVKDYGDLPFADIPNDSPFQIVKNPRSVGKASEQLAGKVAEVKKNGRISLVLGGDHSLAIGSISGHARVHPDLGVIWVDAHTDINTPLTTTSGNLHGQPVSFLLKELKGKIPDVPGFSWVTPSISAKDIVYIGLRDVDPGEHYILKTLGIKYFSMTEVDRLGIGKVMEETLSYLLGRKKRPIHLSFDVDGLDPSFTPATGTPVVGGLTYREGLYITEEIYKTGLLSGLDIMEVNPSLGKTPEEVTRTVNTAVAITLASFGLAREGNHKPIDYLNPPK

SEQ ID NO: 105 - protein, 46 aa, synthetic construct
  REGION 1..46: note = A(EAAAK)4ALEA-(EAAAK)4A Peptide Linker, Synthesized in the Lab
AEAAAKEAAAKEAAAKEAAAKALEAEAAAKEAAAKEAAAKEAAAKA

SEQ ID NO: 106 - protein, 15 aa, synthetic construct
  REGION 1..15: note = G4SG4SG3SG Peptide Linker, Synthesized in the Lab
GGGGSGGGGSGGGSG

SEQ ID NO: 107 - protein, 20 aa, synthetic construct
  REGION 1..20: note = (G4S)n Peptide Linker, Synthesized in the Lab
  REGION 5..20: note = MISC_FEATURE - These amino acids may be absent
GGGGSGGGGSGGGGSGGGGS

SEQ ID NO: 108 - protein, 44 aa, synthetic construct
  REGION 1..44: note = [A(EAAAK)nA]x Peptide Linker, Synthesized in the Lab
  REGION 12..21: note = MISC_FEATURE - These amino acids may be absent
  REGION 23..44: note = MISC_FEATURE - These amino acids may be absent
AEAAAKEAAAKEAAAKEAAAKAAEAAAKEAAAKEAAAKEAAAKA

SEQ ID NO: 109 - protein, 15 aa, synthetic construct
  REGION 1..15: note = (G4S)3 Peptide Linker, Synthesized in the Lab
GGGGSGGGGSGGGGS

SEQ ID NO: 110 - protein, 60 aa, synthetic construct
  REGION 1..60: note = (GS)n, Peptide Synthesized in the Lab
  REGION 3..60: note = MISC_FEATURE - These amino acids may be absent
GSGSGSGSGSGSGSGSGSGSGSGSGSGSGSGSGSGSGSGSGSGSGSGSGSGSGSGSGSGS

SEQ ID NO: 111 - protein, 90 aa, synthetic construct
  REGION 1..90: note = (GGS)n Peptide Linker, Synthesized in the Lab
  REGION 4..90: note = MISC_FEATURE - These amino acids may be absent
GGSGGSGGSGGSGGSGGSGGSGGSGGSGGSGGSGGSGGSGGSGGSGGSGGSGGSGGSGGSGGSGGSGGSGGSGGSGGSGGSGGSGGSGGS

SEQ ID NO: 112 - protein, 15 aa, synthetic construct
  REGION 1..15: note = GS(N)nGSG Peptide Linker, Synthesized in the Lab
  REGION 4..12: note = MISC_FEATURE - These amino acids may be absent
GSNNNNNNNNNNGSG

SEQ ID NO: 113 - protein, 15 aa, synthetic construct
  REGION 1..15: note = GS(Q)nGSG Peptide Linker, Synthesized in the Lab
  REGION 4..12: note = MISC_FEATURE - These amino acids may be absent
GSQQQQQQQQQQGSG